European Patent Application EP 4 729 607 A1, published April 22, 2026. Title: Cell cryopreservation method, cell culture method, and cryopreservation substrate. Applicant: UBE株式会社. The sequence listing filed with the application follows.

SEQUENCE LISTING (4 sequences)

SEQ ID NO: 1 - DNA, 20 bp, synthetic construct
  source 1..20: mol_type = other DNA
ccaacaacaccaactttcac

SEQ ID NO: 2 - DNA, 20 bp, synthetic construct
  source 1..20: mol_type = other DNA
gttgcagacaattcagtgcc

SEQ ID NO: 3 - DNA, 20 bp, synthetic construct
  source 1..20: mol_type = other DNA
acaccagcagcacctagaag

SEQ ID NO: 4 - DNA, 24 bp, synthetic construct
  source 1..24: mol_type = other DNA
ctagtataattttcttggtataag